European Patent Application EP 4 729 548 A2, published April 22, 2026. Title: Materials and Methods for Treating Friedreichs Ataxia. Applicant: The Trustees of Indiana University. Application EP, filed December 19, 2025. The sequence listing filed with the application follows.

SEQUENCE LISTING (11 sequences)

SEQ ID NO: 1 - protein, 224 aa, synthetic construct
  REGION 1..224: note = source = /note="Description of Artificial Sequence: Synthetic polypeptide"
MYGRKKRRQRRRGGMWTLGRRAVAGLLASPSPAQAQTLTRVPRPAELAPLCGRRGLRTDIDATCTPRRASSNQRGLNQIWNVKKQSVYLMNLRKSGTLGHPGSLDETTYERLAEETLDSLAEFFEDLADKPYTFEDYDVSFGSGVLTVKLGGDLGTYVINKQTPNKQIWLSSPSSGPKRYDWTGKNWVYSHDGVSLHELLAAELTKALKTKLDLSSLAYSGKDA

SEQ ID NO: 2 - protein, 12 aa, synthetic construct
  REGION 1..12: note = source = /note="Description of Artificial Sequence: Synthetic peptide"
MYGRKKRRQRRR

SEQ ID NO: 3 - protein, 80 aa, Homo sapiens
MWTLGRRAVAGLLASPSPAQAQTLTRVPRPAELAPLCGRRGLRTDIDATCTPRRASSNQRGLNQIWNVKKQSVYLMNLRK

SEQ ID NO: 4 - protein, 210 aa, Homo sapiens
MWTLGRRAVAGLLASPSPAQAQTLTRVPRPAELAPLCGRRGLRTDIDATCTPRRASSNQRGLNQIWNVKKQSVYLMNLRKSGTLGHPGSLDETTYERLAEETLDSLAEFFEDLADKPYTFEDYDVSFGSGVLTVKLGGDLGTYVINKQTPNKQIWLSSPSSGPKRYDWTGKNWVYSHDGVSLHELLAAELTKALKTKLDLSSLAYSGKDA

SEQ ID NO: 5 - protein, 130 aa, Homo sapiens
SGTLGHPGSLDETTYERLAEETLDSLAEFFEDLADKPYTFEDYDVSFGSGVLTVKLGGDLGTYVINKQTPNKQIWLSSPSSGPKRYDWTGKNWVYSHDGVSLHELLAAELTKALKTKLDLSSLAYSGKDA

SEQ ID NO: 6 - DNA, 684 bp, synthetic construct
  misc_feature 1..684: note = source = /note="Description of Artificial Sequence: Synthetic polynucleotide"
  source 1..684: mol_type = other DNA
catatgtatggtagaaagaaacgtcgtcaacgtcgtcgtggtggtatgtggaccttgggccgtcgcgcggttgcgggcctgctggcgagcccaagcccggcacaggcgcagaccctgacgcgcgttccgcgtccggcggaattggccccgttgtgcggtcgccgtggtctgcgcacggatatcgacgctacctgtacgccgcgtcgcgcgagcagcaatcagcgtggcctgaatcaaatttggaacgtcaagaaacaatctgtttacctgatgaatctgcgcaagagcggtacgttgggtcacccgggcagcctggacgagactacctatgagcgcctggctgaggaaacgctggacagcctggccgaatttttcgaagatctcgcagataagccgtacacgtttgaggattatgacgtgagcttcggcagcggcgtcttaaccgtgaaactgggtggtgacctgggcacctacgtgatcaataagcaaaccccgaacaaacagatttggctgagctcgccgagctctggccctaagcgttacgattggaccggtaagaactgggtgtattcccacgacggtgtcagcctgcatgaactgctggcggcagagctgaccaaagcgctgaaaactaaactggatctgagctccctggcctacagcggtaaagacgcataactcgag

SEQ ID NO: 7 - protein, 11 aa, Human immunodeficiency virus
YGRKKRRQRRR

SEQ ID NO: 8 - protein, 8 aa, synthetic construct
  REGION 1..8: note = source = /note="Description of Artificial Sequence: Synthetic peptide"
GGGGGGGG

SEQ ID NO: 9 - protein, 5 aa, synthetic construct
  REGION 1..5: note = source = /note="Description of Artificial Sequence: Synthetic peptide"
GGGGS

SEQ ID NO: 10 - protein, 12 aa, synthetic construct
  REGION 1..12: note = source = /note="Description of Artificial Sequence: Synthetic peptide"
GSAGSAAGSGEF

SEQ ID NO: 11 - protein, 6 aa, synthetic construct
  REGION 1..6: note = source = /note="Description of Artificial Sequence: Synthetic 6xHis tag"
HHHHHH